European Patent Application EP 4 332 229 A1, published March 6, 2024. Title: Mutant of Corynebacterium glutamicum with enhanced L-lysine productivity and method for preparing L-lysine using the same. Applicant: DAESANG CORPORATION. The sequence listing filed with the application follows.

SEQUENCE LISTING (6 sequences)

SEQ ID NO: 1 - DNA, 134 bp, Artificial Sequence
  promoter sequence of aspB gene
agggtcagcgagctctgacgggtgcgcgggatcccctaaaacgtctagagtagtggcttgaggtcactgctctttttttgtgcccttttttggtccgtctattttgccaccacatgcggaggtacgcagttatg

SEQ ID NO: 2 - DNA, 134 bp, Artificial Sequence
  mutant promoter sequence of aspB gene
agggtcagcgagctctgacgggtgcgcgggatcccctaaaacgtctagagtagtggcttgaggtcactgctctttttttgtgcccttttttggtccgtctattttgccagcacatgcggaggtacgcagttatg

SEQ ID NO: 3 - DNA, 134 bp, Artificial Sequence
  mutant promoter sequence of aspB gene
agggtcagcgagctctgacgggtgcgcgggatcccctaaaacgtctagagtagtggcttgaggtcactgctctttttttgtgccctattttggtccgtctattttgccaccacatgcggaggtacgcagttatg

SEQ ID NO: 4 - DNA, 134 bp, Artificial Sequence
  mutant promoter sequence of aspB gene
agggtcagcgagctctgacgggtgcgcgggatcccctaaaacgactagagtagtggcttgaggtcactgctctttttttgtgcccttttttggtccgtctattttgccaccacatgcggaggtacgcagttatg

SEQ ID NO: 5 - DNA, 18 bp, Artificial Sequence
  DS7-F
cgagaattaccggcgatg

SEQ ID NO: 6 - DNA, 18 bp, Artificial Sequence
  DS7-R
tcaccgtgaaaccagtcg